European Patent Specification EP 4 248 210 B1, published July 1, 2026. Title: HIGH THROUGHPUT DRUG SCREENING METHODS. Applicant: NERD BIO LLC. The sequence listing filed with the application follows.

SEQUENCE LISTING (34 sequences)

SEQ ID NO: 1 - protein, 20 aa, Artificial Sequence
  Description of Artificial Sequence: Synthetic peptide
KETAAAKFERQHMDSSTSAA

SEQ ID NO: 2 - protein, 19 aa, Artificial Sequence
  Description of Artificial Sequence: Synthetic peptide
KETNWAWFWDQHMDSSTSA

SEQ ID NO: 3 - protein, 19 aa, Artificial Sequence
  Description of Artificial Sequence: Synthetic peptide
KETGWALFVQQHMDSSTSA

SEQ ID NO: 4 - protein, 19 aa, Artificial Sequence
  Description of Artificial Sequence: Synthetic peptide
KETVMANFQMQHMDSSTSA

SEQ ID NO: 5 - protein, 19 aa, Artificial Sequence
  Description of Artificial Sequence: Synthetic peptide
KETGDAVFARQHMDSSTSA

SEQ ID NO: 6 - protein, 19 aa, Artificial Sequence
  Description of Artificial Sequence: Synthetic peptide
KETGWAAFVKQHMDSSTSA

SEQ ID NO: 7 - protein, 19 aa, Artificial Sequence
  Description of Artificial Sequence: Synthetic peptide
KETGWATFVEQHMDSSTSA

SEQ ID NO: 8 - protein, 19 aa, Artificial Sequence
  Description of Artificial Sequence: Synthetic peptide
KETKLAFFLKQHMDSSTSA

SEQ ID NO: 9 - protein, 19 aa, Artificial Sequence
  Description of Artificial Sequence: Synthetic peptide
KETWWAWFFGQHMDSSTSA

SEQ ID NO: 10 - protein, 19 aa, Artificial Sequence
  Description of Artificial Sequence: Synthetic peptide
KETTWAEFTWQHMDSSTSA

SEQ ID NO: 11 - protein, 19 aa, Artificial Sequence
  Description of Artificial Sequence: Synthetic peptide
KETPWASFNKQHMDSSTSA

SEQ ID NO: 12 - protein, 19 aa, Artificial Sequence
  Description of Artificial Sequence: Synthetic peptide
KETAMAMFVTQHMDSSTSA

SEQ ID NO: 13 - protein, 19 aa, Artificial Sequence
  Description of Artificial Sequence: Synthetic peptide
KETLWAWFMWQHMDSSTSA

SEQ ID NO: 14 - protein, 15 aa, Artificial Sequence
  Description of Artificial Sequence: Synthetic peptide
KETAAAKFERQHMDS

SEQ ID NO: 15 - protein, 15 aa, Artificial Sequence
  Description of Artificial Sequence: Synthetic peptide
KETAAAKFERQHMNS

SEQ ID NO: 16 - protein, 15 aa, Artificial Sequence
  Description of Artificial Sequence: Synthetic peptide
NRAWSEFLWQHLAPV

SEQ ID NO: 17 - protein, 15 aa, Artificial Sequence
  Description of Artificial Sequence: Synthetic peptide
NRGWSEFLWQHHAPV

SEQ ID NO: 18 - protein, 15 aa, Artificial Sequence
  Description of Artificial Sequence: Synthetic peptide
NRAWSVFQWQHIAPA

SEQ ID NO: 19 - protein, 105 aa, Artificial Sequence
  Description of Artificial Sequence: Synthetic polypeptide
MSSSNYCNQMMKSRNLTKDRCKPVNTFVHESLADVQAVCSQKNVACKNGQTNCYQSYSTMSITDCRETGSSKYPNCAYKTTQANKHIIVACEGNPYVPVHFDASV

SEQ ID NO: 20 - protein, 102 aa, Artificial Sequence
  Description of Artificial Sequence: Synthetic polypeptide
MSSSNYCNQMMKSRNLTKDRCKPVNTFVHESLADVQAVCSQKNVACKNGQTNCYQSYSTMSITDCRETGSSKYPNCAYKTTQANKHIIVACEGNPYVPVHFD

SEQ ID NO: 21 - protein, 124 aa, Bos taurus
KETAAAKFERQHMDSSTSAASSSNYCNQMMKSRNLTKDRCKPVNTFVHESLADVQAVCSQKNVACKNGQTNCYQSYSTMSITDCRETGSSKYPNCAYKTTQANKHIIVACEGNPYVPVHFDASV

SEQ ID NO: 22 - DNA, 348 bp, Artificial Sequence
  Description of Artificial Sequence: Synthetic polynucleotide
ggtaccatgagcagctccaactactgtaaccagatgatgaagagccggaacctgaccaaagatcgatgcaagccagtgaacacctttgtgcacgagtccctggctgatgtccaggccgtgtgctcccagaaaaatgttgcctgcaagaatgggcagaccaattgctaccagagctactccaccatgagcatcaccgactgccgtgagaccggcagctccaagtaccccaactgtgcctacaagaccacccaggcgaataaacacatcattgtggcttgtgagggaaacccgtacgtgccagtccactttgatgcttcagtgcatcaccatcaccatcactagggatcc

SEQ ID NO: 23 - protein, 111 aa, Artificial Sequence
  Description of Artificial Sequence: Synthetic polypeptide
MSSSNYCNQMMKSRNLTKDRCKPVNTFVHESLADVQAVCSQKNVACKNGQTNCYQSYSTMSITDCRETGSSKYPNCAYKTTQANKHIIVACEGNPYVPVHFDASVHHHHHH

SEQ ID NO: 24 - DNA, 552 bp, Artificial Sequence
  Description of Artificial Sequence: Synthetic polynucleotide
ggtaccatgggcgcctccaggctctataccctggtgctggtcctgcagcctcagcgagttctcctgggcatgaaaaagcgaggcttcggggccggccggtggaatggctttgggggcaaagtgcaagaaggagagaccatcgaggatggggctaggagggagctgcaggaggagagcggtctgacagtggacgccctgcacaaggtgggccagatcgtgtttgagttcgtgggcgagcctgagctcatggacgtgcatgtcttctgcacagacagcatccaggggacccccgtggagagcgacgaaatgcgcccatgctggttccagctggatcagatccccttcaaggacatgtggcccgacgacagctactggtttccactcctgcttcagaagaagaaattccacgggtacttcaagttccagggtcaggacaccatcctggactacacactccgcgaggtggacacggtcaaggaaactgcagcagccaagtttgagcggcagcacatggactccagcacttccgctgcctaggctgcctagggatcc

SEQ ID NO: 25 - protein, 176 aa, Artificial Sequence
  Description of Artificial Sequence: Synthetic polypeptide
MGASRLYTLVLVLQPQRVLLGMKKRGFGAGRWNGFGGKVQEGETIEDGARRELQEESGLTVDALHKVGQIVFEFVGEPELMDVHVFCTDSIQGTPVESDEMRPCWFQLDQIPFKDMWPDDSYWFPLLLQKKKFHGYFKFQGQDTILDYTLREVDTVKETAAAKFERQHMDSSTSAA

SEQ ID NO: 26 - DNA, 561 bp, Artificial Sequence
  Description of Artificial Sequence: Synthetic polynucleotide
ggtaccatgggcgcctccaggctctataccctggtgctggtcctgcagcctcagcgagttctcctgggcatgaaaaagcgaggcttcggggccggccggtggaatggctttgggggcaaagtgcaagaaggagagaccatcgaggatggggctaggagggagctgcaggaggagagcggtctgacagtggacgccctgcacaaggtgggccagatcgtgtttgagttcgtgggcgagcctgagctcatggacgtgcatgtcttctgcacagacagcatccaggggacccccgtggagagcgacgaaatgcgcccatgctggttccagctggatcagatccccttcaaggacatgtggcccgacgacagctactggtttccactcctgcttcagaagaagaaattccacgggtacttcaagttccagggtcaggacaccatcctggactacacactccgcgaggtggacacggtcgccgccgccaaggaaactgcagcagccaagtttgagcggcagcacatggactccagcacttccgctgcctaggctgcctagggatcc

SEQ ID NO: 27 - protein, 179 aa, Artificial Sequence
  Description of Artificial Sequence: Synthetic polypeptide
MGASRLYTLVLVLQPQRVLLGMKKRGFGAGRWNGFGGKVQEGETIEDGARRELQEESGLTVDALHKVGQIVFEFVGEPELMDVHVFCTDSIQGTPVESDEMRPCWFQLDQIPFKDMWPDDSYWFPLLLQKKKFHGYFKFQGQDTILDYTLREVDTVAAAKETAAAKFERQHMDSSTSAA

SEQ ID NO: 28 - DNA, 582 bp, Artificial Sequence
  Description of Artificial Sequence: Synthetic polynucleotide
ggtaccatgggcgcctccaggctctataccctggtgctggtcctgcagcctcagcgagttctcctgggcatgaaaaagcgaggcttcggggccggccggtggaatggctttgggggcaaagtgcaagaaggagagaccatcgaggatggggctaggagggagctgcaggaggagagcggtctgacagtggacgccctgcacaaggtgggccagatcgtgtttgagttcgtgggcgagcctgagctcatggacgtgcatgtcttctgcacagacagcatccaggggacccccgtggagagcgacgaaatgcgcccatgctggttccagctggatcagatccccttcaaggacatgtggcccgacgacagctactggtttccactcctgcttcagaagaagaaattccacgggtacttcaagttccagggtcaggacaccatcctggactacacactccgcgaggtggacacggtcgccgccgccgccgccgccgccgccgccgccaaggaaactgcagcagccaagtttgagcggcagcacatggactccagcacttccgctgcctaggctgcctagggatcc

SEQ ID NO: 29 - protein, 186 aa, Artificial Sequence
  Description of Artificial Sequence: Synthetic polypeptide
MGASRLYTLVLVLQPQRVLLGMKKRGFGAGRWNGFGGKVQEGETIEDGARRELQEESGLTVDALHKVGQIVFEFVGEPELMDVHVFCTDSIQGTPVESDEMRPCWFQLDQIPFKDMWPDDSYWFPLLLQKKKFHGYFKFQGQDTILDYTLREVDTVAAAAAAAAAAKETAAAKFERQHMDSSTSAA

SEQ ID NO: 30 - DNA, 2181 bp, Artificial Sequence
  Description of Artificial Sequence: Synthetic polynucleotide
atggcctcgccggctgacagctgtatccagttcacccgccatgccagtgatgttcttctcaaccttaatcgtctccggagtcgagacatcttgactgatgttgtcattgttgtgagccgtgagcagtttagagcccataaaacggtcctcatggcctgcagtggcctgttctatagcatctttacagaccagttgaaatgcaaccttagtgtgatcaatctagatcctgagatcaaccctgagggattctgcatcctcctggacttcatgtacacatctcggctcaatttgcgggagggcaacatcatggctgtgatggccacggctatgtacctgcagatggagcatgttgtggacacttgccggaagtttattaaggccagtgaagcagagatggtttctgccatcaagcctcctcgtgaagagttcctcaacagccggatgctgatgccccaagacatcatggcctatcggggtcgtgaggtggtggagaacaacctgccactgaggagcgcccctgggtgtgagagcagagcctttgcccccagcctgtacagtggcctgtccacaccgccagcctcttattccatgtacagccacctccctgtcagcagcctcctcttctccgatgaggagtttcgggatgtccggatgcctgtggccaaccccttccccaaggagcgggcactcccatgtgatagtgccaggccagtccctggtgagtacagccggccgactttggaggtgtcccccaatgtgtgccacagcaatatctattcacccaaggaaacaatcccagaagaggcacgaagtgatatgcactacagtgtggctgagggcctcaaacctgctgccccctcagcccgaaatgccccctacttcccttgtgacaaggccagcaaagaagaagagagaccctcctcggaagatgagattgccctgcatttcgagccccccaatgcacccctgaaccggaagggtctggttagtccacagagcccccagaaatctgactgccagcccaactcgcccacagagtcctgcagcagtaagaatgcctgcatcctccaggcttctggctcccctccagccaagagccccactgaccccaaagcctgcaactggaagaaatacaagttcatcgtgctcaacagcctcaaccagaatgccaaaccagaggggcctgagcaggctgagctgggccgcctttccccacgagcctacacggccccacctgcctgccagccacccatggagcctgagaaccttgacctccagtccccaaccaagctgagtgccagcggggaggactccaccatcccacaagccagccggctcaataacatcgttaacaggtccatgacgggctctccccgcagcagcagcgagagccactcaccactctacatgcaccccccgaagtgcacgtcctgcggctctcagtccccacagcatgcagagatgtgcctccacaccgctggccccacgttccctgaggagatgggagagacccagtctgagtactcagattctagctgtgagaacggggccttcttctgcaatgagtgtgactgccgcttctctgaggaggcctcactcaagaggcacacgctgcagacccacagtgacaaaccctacaagtgtgaccgctgccaggcctccttccgctacaagggcaacctcgccagccacaagaccgtccataccggtgagaaaccctatcgttgcaacatctgtggggcccagttcaaccggccagccaacctgaaaacccacactcgaattcactctggagagaagccctacaaatgcgaaacctgcggagccagatttgtacaggtggcccacctccgtgcccatgtgcttatccacactggtgagaagccctatccctgtgaaatctgtggcacccgtttccggcaccttcagactctgaagagccacctgcgaatccacacaggagagaaaccttaccattgtgagaagtgtaacctgcatttccgtcacaaaagccagctgcgacttcacttgcgccagaagcatggcgccatcaccaacaccaaggtgcaataccgcgtgtcagccactgacctgcctccggagctccccaaagcctgcaaggaaactgcagcagccaagtttgagcggcagcacatggactccagcacttccgctgcctga

SEQ ID NO: 31 - protein, 726 aa, Artificial Sequence
  Description of Artificial Sequence: Synthetic polypeptide
MASPADSCIQFTRHASDVLLNLNRLRSRDILTDVVIVVSREQFRAHKTVLMACSGLFYSIFTDQLKCNLSVINLDPEINPEGFCILLDFMYTSRLNLREGNIMAVMATAMYLQMEHVVDTCRKFIKASEAEMVSAIKPPREEFLNSRMLMPQDIMAYRGREVVENNLPLRSAPGCESRAFAPSLYSGLSTPPASYSMYSHLPVSSLLFSDEEFRDVRMPVANPFPKERALPCDSARPVPGEYSRPTLEVSPNVCHSNIYSPKETIPEEARSDMHYSVAEGLKPAAPSARNAPYFPCDKASKEEERPSSEDEIALHFEPPNAPLNRKGLVSPQSPQKSDCQPNSPTESCSSKNACILQASGSPPAKSPTDPKACNWKKYKFIVLNSLNQNAKPEGPEQAELGRLSPRAYTAPPACQPPMEPENLDLQSPTKLSASGEDSTIPQASRLNNIVNRSMTGSPRSSSESHSPLYMHPPKCTSCGSQSPQHAEMCLHTAGPTFPEEMGETQSEYSDSSCENGAFFCNECDCRFSEEASLKRHTLQTHSDKPYKCDRCQASFRYKGNLASHKTVHTGEKPYRCNICGAQFNRPANLKTHTRIHSGEKPYKCETCGARFVQVAHLRAHVLIHTGEKPYPCEICGTRFRHLQTLKSHLRIHTGEKPYHCEKCNLHFRHKSQLRLHLRQKHGAITNTKVQYRVSATDLPPELPKACKETAAAKFERQHMDSSTSAA

SEQ ID NO: 32 - DNA, 3693 bp, Artificial Sequence
  Description of Artificial Sequence: Synthetic polynucleotide
atgcgaccctccgggacggccggggcagcgctcctggcgctgctggctgcgctctgcccggcgagtcgggctctggaggaaaagaaagtttgccaaggcacgagtaacaagctcacgcagttgggcacttttgaagatcattttctcagcctccagaggatgttcaataactgtgaggtggtccttgggaatttggaaattacctatgtgcagaggaattatgatctttccttcttaaagaccatccaggaggtggctggttatgtcctcattgccctcaacacagtggagcgaattcctttggaaaacctgcagatcatcagaggaaatatgtactacgaaaattcctatgccttagcagtcttatctaactatgatgcaaataaaaccggactgaaggagctgcccatgagaaatttacaggaaatcctgcatggcgccgtgcggttcagcaacaaccctgccctgtgcaacgtggagagcatccagtggcgggacatagtcagcagtgactttctcagcaacatgtcgatggacttccagaaccacctgggcagctgccaaaagtgtgatccaagctgtcccaatgggagctgctggggtgcaggagaggagaactgccagaaactgaccaaaatcatctgtgcccagcagtgctccgggcgctgccgtggcaagtcccccagtgactgctgccacaaccagtgtgctgcaggctgcacaggcccccgggagagcgactgcctggtctgccgcaaattccgagacgaagccacgtgcaaggacacctgccccccactcatgctctacaaccccaccacgtaccagatggatgtgaaccccgagggcaaatacagctttggtgccacctgcgtgaagaagtgtccccgtaattatgtggtgacagatcacggctcgtgcgtccgagcctgtggggccgacagctatgagatggaggaagacggcgtccgcaagtgtaagaagtgcgaagggccttgccgcaaagtgtgtaacggaataggtattggtgaatttaaagactcactctccataaatgctacgaatattaaacacttcaaaaactgcacctccatcagtggcgatctccacatcctgccggtggcatttaggggtgactccttcacacatactcctcctctggatccacaggaactggatattctgaaaaccgtaaaggaaatcacagggtttttgctgattcaggcttggcctgaaaacaggacggacctccatgcctttgagaacctagaaatcatacgcggcaggaccaagcaacatggtcagttttctcttgcagtcgtcagcctgaacataacatccttgggattacgctccctcaaggagataagtgatggagatgtgataatttcaggaaacaaaaatttgtgctatgcaaatacaataaactggaaaaaactgtttgggacctccggtcagaaaaccaaaattataagcaacagaggtgaaaacagctgcaaggccacaggccaggtctgccatgccttgtgctcccccgagggctgctggggcccggagcccagggactgcgtctcttgccggaatgtcagccgaggcagggaatgcgtggacaagtgcaaccttctggagggtgagccaagggagtttgtggagaactctgagtgcatacagtgccacccagagtgcctgcctcaggccatgaacatcacctgcacaggacggggaccagacaactgtatccagtgtgcccactacattgacggcccccactgcgtcaagacctgcccggcaggagtcatgggagaaaacaacaccctggtctggaagtacgcagacgccggccatgtgtgccacctgtgccatccaaactgcacctacggatgcactgggccaggtcttgaaggctgtccaacgaatgggcctaagatcccgtccatcgccactgggatggtgggggccctcctcttgctgctggtggtggccctggggatcggcctcttcatgcgaaggcgccacatcgttcggaagcgcacgctgcggaggctgctgcaggagagggagcttgtggagcctcttacacccagtggagaagctcccaaccaagctctcttgaggatcttgaaggaaactgaattcaaaaagatcaaagtgctgggctccggtgcgttcggcacggtgtataagggactctggatcccagaaggtgagaaagttaaaattcccgtcgctatcaaggaattaagagaagcaacatctccgaaagccaacaaggaaatcctcgatgaagcctacgtgatggccagcgtggacaacccccacgtgtgccgcctgctgggcatctgcctcacctccaccgtgcagctcatcatgcagctcatgcccttcggctgcctcctggactatgtccgggaacacaaagacaatattggctcccagtacctgctcaactggtgtgtgcagatcgcaaagggcatgaactacttggaggaccgtcgcttggtgcaccgcgacctggcagccaggaacgtactggtgaaaacaccgcagcatgtcaagatcacagattttgggcgggccaaactgctgggtgcggaagagaaagaataccatgcagaaggaggcaaagtgcctatcaagtggatggcattggaatcaattttacacagaatctatacccaccagagtgatgtctggagctacggggtgactgtttgggagttgatgacctttggatccaagccatatgacggaatccctgccagcgagatctcctccatcctggagaaaggagaacgcctccctcagccacccatatgtaccatcgatgtctacatgatcatggtcaagtgctggatgatagacgcagatagtcgcccaaagttccgtgagttgatcatcgaattctccaaaatggcccgagacccccagcgctaccttgtcattcagggggatgaaagaatgcatttgccaagtcctacagactccaacttctaccgtgccctgatggatgaagaagacatggacgacgtggtggatgccgacgagtacctcatcccacagcagggcttcttcagcagcccctccacgtcacggactcccctcctgagctctctgagtgcaaccagcaacaattccaccgtggcttgcattgatagaaatgggctgcaaagctgtcccatcaaggaagacagcttcttgcagcgatacagctcagaccccacaggcgccttgactgaggacagcatagacgacaccttcctcccagtgcctgaatacataaaccagtccgttcccaaaaggcccgctggctctgtgcagaatcctgtctatcacaatcagcctctgaaccccgcgcccagcagagacccacactaccaggacccccacagcactgcagtgggcaaccccgagtatctcaacactgtccagcccacctgtgtcaacagcacattcgacagccctgcccactgggcccagaaaggcagccaccaaattagcctggacaaccctgactaccagcaggacttctttcccaaggaagccaagccaaatggcatctttaagggctccacagctgaaaatgcagaatacctaagggtcgcgccacaaagcagtgaatttattggagcaaaggaaactgcagcagccaagtttgagcggcagcacatggactccagcacttccgctgcctga

SEQ ID NO: 33 - protein, 1230 aa, Artificial Sequence
  Description of Artificial Sequence: Synthetic polypeptide
MRPSGTAGAALLALLAALCPASRALEEKKVCQGTSNKLTQLGTFEDHFLSLQRMFNNCEVVLGNLEITYVQRNYDLSFLKTIQEVAGYVLIALNTVERIPLENLQIIRGNMYYENSYALAVLSNYDANKTGLKELPMRNLQEILHGAVRFSNNPALCNVESIQWRDIVSSDFLSNMSMDFQNHLGSCQKCDPSCPNGSCWGAGEENCQKLTKIICAQQCSGRCRGKSPSDCCHNQCAAGCTGPRESDCLVCRKFRDEATCKDTCPPLMLYNPTTYQMDVNPEGKYSFGATCVKKCPRNYVVTDHGSCVRACGADSYEMEEDGVRKCKKCEGPCRKVCNGIGIGEFKDSLSINATNIKHFKNCTSISGDLHILPVAFRGDSFTHTPPLDPQELDILKTVKEITGFLLIQAWPENRTDLHAFENLEIIRGRTKQHGQFSLAVVSLNITSLGLRSLKEISDGDVIISGNKNLCYANTINWKKLFGTSGQKTKIISNRGENSCKATGQVCHALCSPEGCWGPEPRDCVSCRNVSRGRECVDKCNLLEGEPREFVENSECIQCHPECLPQAMNITCTGRGPDNCIQCAHYIDGPHCVKTCPAGVMGENNTLVWKYADAGHVCHLCHPNCTYGCTGPGLEGCPTNGPKIPSIATGMVGALLLLLVVALGIGLFMRRRHIVRKRTLRRLLQERELVEPLTPSGEAPNQALLRILKETEFKKIKVLGSGAFGTVYKGLWIPEGEKVKIPVAIKELREATSPKANKEILDEAYVMASVDNPHVCRLLGICLTSTVQLIMQLMPFGCLLDYVREHKDNIGSQYLLNWCVQIAKGMNYLEDRRLVHRDLAARNVLVKTPQHVKITDFGRAKLLGAEEKEYHAEGGKVPIKWMALESILHRIYTHQSDVWSYGVTVWELMTFGSKPYDGIPASEISSILEKGERLPQPPICTIDVYMIMVKCWMIDADSRPKFRELIIEFSKMARDPQRYLVIQGDERMHLPSPTDSNFYRALMDEEDMDDVVDADEYLIPQQGFFSSPSTSRTPLLSSLSATSNNSTVACIDRNGLQSCPIKEDSFLQRYSSDPTGALTEDSIDDTFLPVPEYINQSVPKRPAGSVQNPVYHNQPLNPAPSRDPHYQDPHSTAVGNPEYLNTVQPTCVNSTFDSPAHWAQKGSHQISLDNPDYQQDFFPKEAKPNGIFKGSTAENAEYLRVAPQSSEFIGAKETAAAKFERQHMDSSTSAA

SEQ ID NO: 34 - protein, 6 aa, Artificial Sequence
  Description of Artificial Sequence: Synthetic 6xHis tag
HHHHHH